European Patent Specification EP 3 708 660 B1, published April 29, 2026. Title: Polypeptides. Applicant: Novozymes A/S Gjermansen, Morten. The sequence listing filed with the application follows.

SEQUENCE LISTING (21 sequences)

SEQ ID NO: 1 - protein, 122 aa, Paenibacillus sp-62212
ETEPTTQQAAGSTSAETITLYFPQDRFPETGKHIKNAIASGESSICTIDRKQAEENRKHSLKGIPTKKGYDRDEWPMAMCAEGGTGADIAYISPSDNRGAGSWVSNQLEKYEDGTKILFIVK

SEQ ID NO: 2 - protein, 118 aa, Paenibacillus sp-62605
NDTSVTTSSTEADVKIVFPSDRFPETAKHIKDAIAAGESPICTIDRDGAEENRKESLKGIATKKGYDRDEWPMAMCAEGGAGADIAYITPSDNRGAGSWVGNQLEKYTDGTRVEFVVE

SEQ ID NO: 3 - protein, 115 aa, BACILLUS SP-62738
SETADSKGYDQVVELPADKYPETAAHIKNAIAKGKTDMCTIDRKGAKDRRKQSLAHIPTKKGYDRDEFPMAFCKEGGSGADIEYISPEDNRGAGSYIGNKVENLKDGTRVKIAVN

SEQ ID NO: 4 - protein, 120 aa, Bacillus pumilus
QLEQSKQETTNSSYDKTIHFPSDRYPETAKHIEEAIDEGHSSVCTIDRKHSDEQRDQSLHGIPTKRGYDRDEWPMAMCKEGGTGASVKYISPSDNRGAGSWVGHQLSDDPDGTRIQFIID

SEQ ID NO: 5 - protein, 249 aa, Bacillus horikoshii
VEDGSSTQLANNSTNHEPSIKVREETETNIEENHEFPRTEVPLIRVIDGDTIKVKIDGKEENVRFLLVDTPETSHPRMNGPQPFGPEAKEFMEEFAATGKLELELDVSERDRYGRVLAYVYVNGVSAQEELLKRGLARVAYIYPPNTRYVDHYQALQEKAQADGVGIWSVENYAQDDGFYPEYVEDPDLKESTEKQPVTENCPVKGNISSSGEKIYHVKTGAFYERTIPEECFNTEEEAMKAGYRKSKR

SEQ ID NO: 6 - protein, 245 aa, Bacillus sp-62490
STYEETKPSSTVETDEIEVDETQKEEIIEETSESFIQATVVRVVDGDTVIVKLPNNQEERVRLLLVDTPESVHPTKPVQPFGIESSEFAKQLMYPGKTVELELDINERDKYGRLLAYVWVGEKMLNELLLEKGLARVAYIFAPNTRHVDRFLEIQKKAQQQELGIWSIENYATESGFAEEAVLEKQEPTKLTKACDDPKIKGNHSSSGELIYHIPGGQYYEKTNPEEMFCTEDEALEAGYRKSMR

SEQ ID NO: 7 - protein, 223 aa, Bacillus sp-13390
KESNSKEAVEQRFIQASVVRVVDGDTLIVKLDHKKEERVRLLLIDTPESVHPDKPVQPFGIEASEMVKELMKPGDLIHLELDVSERDKYGRLLAYVWIEDKMVNELLLEKGFARVAYVYAPNTKYVDQFYDIQKQAQERGIGIWSLENYVVDRGFNEEVYLEKDNPSHSDLSCSNPMIKGNHSSRGDFIYHVPEGQYYDQTNAEEMFCTEEEAKAAGYRKSMK

SEQ ID NO: 8 - protein, 210 aa, Jeotgalibacillus sp-13376
DKPERLNAVVTNVVDGDTIDVKTEDGSIERVRLLLIDTPETKHPQMGVQPFGHEASIYTESALLGEKIQLEFDVSERDRYGRVLAYIWHQDELFNQTLIEKGLARVSIYPPDIKYVDEFEKIQEEARKSELGIWSLQNYVTKKGYERKLDQSKDEEIIQPDGCTIKGNINSKGEKIYHDTNSRSYSQTIPEEWFCTIEEAKAAGFRAPRN

SEQ ID NO: 9 - protein, 231 aa, Bacillus sp-62738
STNKQEPSQATTKQESNQTQNKTSNGQQQSYNIEDIAKNYKGQKVVEINGNKADFTQDQLDKVQLKNTNPTWQEFSNLDSKNRVGVATALIGKEIQPKEKRDERLNTKPTGWHQKKLSDGSTLFDRSHLIGYQLTGQNDNPKNLMTGTKDFNRHSMLKYENMVDKEVEKGSYVLYEVKPVFIGDELVARGVQMKAKTVNNNHLDFNVFCFNVQDGVEIDYKDGTSKLVNKQ

SEQ ID NO: 10 - protein, 268 aa, Streptomyces iakyrus
RSLLDLLKPPTQHQEQTSRSGSISQSAALDLYSNQQKQASFDGCAELFPAAKPINVATVPATMNPMALCSDNFAVLYSQTSKTPLIVVERLNASQLQDAKGEERTNQFYPDPRIPKSGRAELSDYRGQHPAVDRGHQSPAADAPNPNAMAQSFALSNMVPQDPTNNRKIWSKVESDVRKFAKRADGNVFVFTGPLFDSGHSTIGENKVWVPTRLFKLVYDASSKRAWAYVLPNAETRIEKPMDYDAFVKSTGLKLLGNLPISGSVGRT

SEQ ID NO: 11 - protein, 245 aa, Streptococcus infantis
SNATPQTQVNQKSQSLDTPSQKLAESVLTDSVKKQIKGTLEWNGSGAFIVNGNKTNLDAKVSSKPYADNKTKTVGGETVPTVANALMSKATRQYKDREETGNGSTSWTPAGWHQVKNLKGTYNHAVDRGHLLGYALIGGLDGFDASTSNPKNIAVQTAWANQARAEDSTGQNYYESLVRKALDQNKRVRYRVTLLYATEEDLVPSASQIEAKSSDGELEFNVVVPNVQKGIQLDYRTGKVTVTKN

SEQ ID NO: 12 - protein, 110 aa, Bacillus sp-62599
ASSYDATLTFPSDKYPYTADHIRDAIAAGQSSICTIDRDGAEQNREESLRGIPTKKGYDRDEWPMAMCEEGGAGADVRYVPSSDNRGSGAWVGNQLSKYPDGTRVKFYVP

SEQ ID NO: 13 - protein, 251 aa, Bacillus akibai
STDENKEDILIETSSAVETDEVEVDEQEHKEESPEESNGTFIQATVVRVVDGDTVIVKLPNNTEERVRLLLIDTPESVHPTKPVQPFGLEASEFAKELMYPGKTVELELDINERDRYGRLLAYVWIGDEMLNELLLENGLARVAYIFAPNTRHVDRFYEIQKKAQQQAIGIWSIENYATEGGFAEEVDLEKQEPSKLANACDDPKIKGNHSSSGDLIYHIPGGQYYEKTNPEEMFCTEEEAKEAGYRKSMR

SEQ ID NO: 14 - protein, 125 aa, Paenibacillus xylanexedens
GGEWPEEIPNPFGGTNKSVDHTITFPSERYPETAKHIKAAIKAGHSDVCTIDRNGAEGNRDLSLKGVPVKKGKDRDEWPMAMCAEGGTGADIQYITPKDNRGAGSWVGNQLSTYPDGTRVKFVVK

SEQ ID NO: 15 - protein, 182 aa, Fictibacillus sp-62719
LPPGTPTKSAAQSQLNALVVKTEGTMTGYSRDLFPHWSSQGGGCDTRQVVLKRDADSFSGNCPVTSGSWYSYYDGITITNPSDLDIDHVVPLAEAWRSGASSWTTDRREAFANDLTGPQLIAVTASSNRSKGDQDPSTWKPTRTAAGCGYAKWWIQTKYNWGLNLQSAEKTSLQSMLNTCTY

SEQ ID NO: 16 - protein, 182 aa, Bacillus algicola
FPPGTPSKSEAQSQLNSLTVQSEGSMSGYSRDKFPHWIGQGNGCDTRQLVLQRDADYYSGDCPVTSGKWYSYFDGVTVYDPSDLDIDHMVPMAEAWRSGASSWSTQKREDFANDLSGPHLIAVTASSNRSKGDQDPSTWKPTRYGAHCGYAKWWINTKYVYDLTLQSSEKTELQSMLNTCSY

SEQ ID NO: 17 - protein, 182 aa, Exiguobacterium sp. NG55
FPPNIPSKADALTKLNALTVKNEGSMTGYSRDIFPHWSSQGSGCNTRHIVLKRDADSVVDQCPVTTGSWYSYYDGLTFTSASDIDIDHVVPLAEAWRSGASSWTTTKRQSFANDLNGPQLIAVSASSNRSKGDQDPSTWQPPRTGARCAYAKMWVETKSRWGLSLQSAEKSALTTAINACSY

SEQ ID NO: 18 - protein, 182 aa, Metagenome from environmental sample J
LPPNIPSKADALTKLNALTVQTEGPMTGYSRDLFPHWSSQGNGCNTRHVVLKRDADSVVDTCPVTTGRWYSYYDGLVFTSASDIDIDHVVPLAEAWRSGASSWTSTKRQSFANDLNGPQLIAVSATSNRSKGDQDPSTWQPPRAGARCAYAKMWVETKSRWGLTLQSSEKAALQTAINACSY

SEQ ID NO: 19 - protein, 216 aa, Streptomyces thermoalcalitolerans
CTEDTGGPGTPEKTAAGAALAAVEELPVKGRAPKTGYEREKFGRAWADTDSNGCRTRDDILKRDLEQVRFTDGTCKVSYGVLASDPYSGKEIVFRRGHSQIDIDHVVALSDAWQKGAKYWDASKRIALANDPLNLLAVDARTNRAKGDGDTATWLPPNKAYRCQYVARQVAVKKKYELWVTAAEKAAMKRVLSTCPDQKLPSGGTPTKAPERFRAQ

SEQ ID NO: 20 - protein, 200 aa, Metagenome from environmental sample C
SLPDYASPISTPTSGLATPASDASPSDRKDRTDYDYELVFPSDKYPETALHIHGAIEMGYSDVCTIDRGGAEQNRKESLAGIETRQGYDRDEWPMAMCGEGGAGASVAYIDAGDNRGAGSWVGNQLKEYPDGTRILFIVDKPANLFPAQSPNASSQPADDAEVYYKNCTAVREAGKAPLHKGEPGYAAHLDRDGNGVACE

SEQ ID NO: 21 - protein, 27 aa, Artificial
  Bacillus clausii secretion signal
MKKPLGKIVASTALLISVAFSSSIASA